European Patent Application EP 4 223 879 A1, published August 9, 2023. Title: ALPHA-AMYLASE VARIANT. Applicant: KAO CORPORATION. The sequence listing filed with the application follows.

SEQUENCE LISTING (4 sequences)

SEQ ID NO: 1 - DNA, 1458 bp, Bacillus sp. YR288
  CDS (1)..(1455): Codon-optimized oligonucleotide
gcagctcaaaacggtacgatgatgcagtactttgaatggtatgtaccgaatgatggtcagcattggaatcgtctgcggaacgatgcagcctacttgaaatccatcggtgtgtcagctatctggacacctcctgcttacaaaggcacaagccagaacgatgttggctatggagcatatgacctgtacgatttaggagaattcaaccagaaaggcactattcgcaccaaatatggaacgaaagctgaactgaaaagcgcggtatcgactctcaagtctaatgggattcaagtgtatggagatgtcgtcatgaatcataaaggcggtgccgattacacagagaatgtaacagctgtggaagtcaatccgagcaatcgcaatcaagaaacatccgatgagtatacgatccaagcatggacaggattcaacttccctgggcgaggcacaacccatagtccgtttaagtggcagtggtatcattttgatggaactgactgggatcagtctcggaatgcgagcagaatcttcaaatttcgtgggacaggaaaagcatgggattgggaagtatcatcggagaatgggaattacgactatcttatgtacgccgatttagactttgatcatcctgatgttagaaatgagatgaagaattggggcgtgtggtacgcgaatgaagttggcttggacggatttaggctggatgcggttaagcacataaagcatagctatctgggcgattgggtgaaccatgtcagaactaagacgggaaaagagatgtttacagttgctgaatattggcaaaacgacgtcaatgccattaataactatttagccaaagtgaactataatcactctgtctttgatgcgcctttgcattacaactttcactatgcaagccagtcaggaggtaactacgacatgcgtaacttattgaacggcacagtcgtggctgctcatccgacaaaagcagttacccttgtcgaaaatcatgacagtcaaccgggacaatctctggagtcagtcgttcaaccgtggtttaagccccttgcctatgcgtttatcctcacacgagcagaaggttatccaagtatcttttatggggatatgtatgggactaagggaaactcatcgtacgaaattccagcactcaaaaccaaaattgaaccgttactgaaagcacgcaaggattatgcctatggtacgcagcacaactatatggaccactgggatgttataggttggaccagagaaggtgactccacgaaagaaaaatctggccttgcgacgcttgtgacagacggggcaggcgggtctaaatggatgtatgtaggcaaacagaatgctggcgaagtttggtatgacatcacaggcaatagaacggataaaatcaccattaatacagatggctggggaaacttccaagtaaacggaggctcagtctccgtgtacgttcaacagtaa

SEQ ID NO: 2 - protein, 485 aa, Bacillus sp. YR288
AAQNGTMMQYFEWYVPNDGQHWNRLRNDAAYLKSIGVSAIWTPPAYKGTSQNDVGYGAYDLYDLGEFNQKGTIRTKYGTKAELKSAVSTLKSNGIQVYGDVVMNHKGGADYTENVTAVEVNPSNRNQETSDEYTIQAWTGFNFPGRGTTHSPFKWQWYHFDGTDWDQSRNASRIFKFRGTGKAWDWEVSSENGNYDYLMYADLDFDHPDVRNEMKNWGVWYANEVGLDGFRLDAVKHIKHSYLGDWVNHVRTKTGKEMFTVAEYWQNDVNAINNYLAKVNYNHSVFDAPLHYNFHYASQSGGNYDMRNLLNGTVVAAHPTKAVTLVENHDSQPGQSLESVVQPWFKPLAYAFILTRAEGYPSIFYGDMYGTKGNSSYEIPALKTKIEPLLKARKDYAYGTQHNYMDHWDVIGWTREGDSTKEKSGLATLVTDGAGGSKWMYVGKQNAGEVWYDITGNRTDKITINTDGWGNFQVNGGSVSVYVQQ

SEQ ID NO: 3 - DNA, 1452 bp, Artificial Sequence
  Synthetic oligonucleotide
  CDS (1)..(1449)
gcagctcaaaacggtacgatgatgcagtactttgaatggtatgtaccgaatgatggtcagcattggaatcgtctgcggaacgatgcagcctacttgaaatccatcggtgtgtcagctatctggacacctcctgcttacaaaggcacaagccagaacgatgttggctatggagcatatgacctgtacgatttaggagaattcaaccagaaaggcactattcgcaccaaatatggaacgaaagctgaactgaaaagcgcggtatcgactctcaagtctaatgggattcaagtgtatggagatgtcgtcatgaatcataaaggcggtgccgattacacagagaatgtaacagctgtggaagtcaatccgagcaatcgcaatcaagaaacatccgatgagtatacgatccaagcatggacaggattcaacttccctgggcgaggcacaacccatagtccgtttaagtggcagtggtatcattttgatggaactgactgggatcagtctcggaatgcgagcagaatcttcaaatttgggggaaaagcatgggattgggaagtatcatcggagaatgggaattacgactatcttatgtacgccgatttagactttgatcatcctgatgttagaaatgagatgaagaattggggcgtgtggtacgcgaatgaagttggcttggacggatttaggctggatgcggttaagcacataaagcatagctatctgggcgattgggtgaaccatgtcagaactaagacgggaaaagagatgtttacagttgctgaatattggcaaaacgacgtcaatgccattaataactatttagccaaagtgaactataatcactctgtctttgatgcgcctttgcattacaactttcactatgcaagccagtcaggaggtaactacgacatgcgtaacttattgaacggcacagtcgtggctgctcatccgacaaaagcagttacccttgtcgaaaatcatgacagtcaaccgggacaatctctggagtcagtcgttcaaccgtggtttaagccccttgcctatgcgtttatcctcacacgagcagaaggttatccaagtatcttttatggggatatgtatgggactaagggaaactcatcgtacgaaattccagcactcaaaaccaaaattgaaccgttactgaaagcacgcaaggattatgcctatggtacgcagcacaactatatggaccactgggatgttataggttggaccagagaaggtgactccacgaaagaaaaatctggccttgcgacgcttgtgacagacggggcaggcgggtctaaatggatgtatgtaggcaaacagaatgctggcgaagtttggtatgacatcacaggcaatagaacggataaaatcaccattaatacagatggctggggaaacttccaagtaaacggaggctcagtctccgtgtacgttcaacagtaa

SEQ ID NO: 4 - protein, 483 aa, Artificial Sequence
  Synthetic Construct
AAQNGTMMQYFEWYVPNDGQHWNRLRNDAAYLKSIGVSAIWTPPAYKGTSQNDVGYGAYDLYDLGEFNQKGTIRTKYGTKAELKSAVSTLKSNGIQVYGDVVMNHKGGADYTENVTAVEVNPSNRNQETSDEYTIQAWTGFNFPGRGTTHSPFKWQWYHFDGTDWDQSRNASRIFKFGGKAWDWEVSSENGNYDYLMYADLDFDHPDVRNEMKNWGVWYANEVGLDGFRLDAVKHIKHSYLGDWVNHVRTKTGKEMFTVAEYWQNDVNAINNYLAKVNYNHSVFDAPLHYNFHYASQSGGNYDMRNLLNGTVVAAHPTKAVTLVENHDSQPGQSLESVVQPWFKPLAYAFILTRAEGYPSIFYGDMYGTKGNSSYEIPALKTKIEPLLKARKDYAYGTQHNYMDHWDVIGWTREGDSTKEKSGLATLVTDGAGGSKWMYVGKQNAGEVWYDITGNRTDKITINTDGWGNFQVNGGSVSVYVQQ